European Patent Specification EP 3 562 944 B1, published July 10, 2024. Title: TRANSGENIC ANIMALS AND METHOD FOR BIOPRODUCTION. Applicant: Applied StemCell, Inc The Regents of the University of Michigan. The sequence listing filed with the application follows.

SEQUENCE LISTING (17 sequences)

SEQ ID NO: 1 - DNA, 23 bp, Artificial Sequence
  Synthetic
ggatatcatgttagagtgcctgg

SEQ ID NO: 2 - DNA, 2990 bp, Oryctolagus cuniculus
gtaagaattctaggtatgaatttcatttactcacccaacctttatttcagaatatgattaaaatacagtttttgaaataaagttacctaagatagtactaaaattatttttaacacttagaaaaaataggatgcctagaaatatttaacaaaacatacaaagatcatataggccttgtaaatcctatgcaatgtagtaactaatttaatatgtgtagcaaaactagctaatacttaatattaagatgatatctatttcttgaattaaatgtcttcaaatttacataacatattaaaaccataaaacaaatatatttaaattagcttgagaagatgaataattattgggaaagttttttttaccaatatgtagcatgctgagtcaagaaacagatggagggagtgggaacatacaatatcctaaatattcataaactttttagaagaagagtgtactcattaaagttaagttgcctagactctccagtttcccagtttatcatctagtttataatatttcaaaataatcttacaatggagacatggagatacagagttaagctgaaaaatcaaattattctacattttaagaaaattctacatgcgacaaagatgtcttgcaaacaaaacacaaaggaaatagatgatttgaaaacagtagatgtataccagtctataataaaattcttgcttaaaaactagtatacaaaatactacgtttaagagatagaaaatgcagtgagattcttcttactttacttgtttattgccttgtgttacatttttttgaactctttacaagaaaaactcctttggaaatttatggtgtctcaggcaaggtaaaattaataaataattataaaccattcataagaaaaacaaaaaattattttcacaaatggaattatttcaaccttcaactattggaaaggatatttttcttttttttttaagattcattttatttatcagaagggcagagtttcagagagagaggaagggaaagacacagagagaggtcttctttctgttggttcactccccaaatagctacaatggccagggttgggccaggccaaagccaggaatcaagagcttctcctgggtctccaatgtgggtgcaggggtccaagcacttggaccttcctccactgctttcccagggcattagcatggagctggattggaagtggagcagtggggacttaaacctgcatccatgtgggatgcccatgctgcatgtagaggcttaacccaccatgccacagcactgggcccaggagatgacagttttcagaagcagaactttattctgagaactgtttgaatttcagaaatttagtttaaaaatatgaaaatgaagatcgagtgtcaaatattattatggcataaaaattaatttttaaaataaatgatttaaaatgcaagaaaaaggaaggatatttggcttagtggttaaagtgctccttaggatatcatgttagagtgcctggctttgagtcctaatgctgctccaactccagcttcctgctaatgcacagcctgagaggcaacaggtaatggctcaactagttggatacctgtcacccaggtgggaggcctgcagtgagttcacagctcttgaatttgttctgacccagccccagcctttgctggcatttggggagtgatccaacagataggagttctctaactgcctttctgtcttgtgtatgtctctctgtctttcagataaaaaaaaaattaaaaatgcaacaagaaaatcatagaggtcatttagtatattttgatcaaaagtattaacatatatttcataagaggtagcttggggttagggagtaggcaagaggaagtagccctttgtaagtcatcaagggatcagtgtgcattttaatagcaagagaaggcctgcgctgcagctcactaggctaatcctccgccttgcggcaccggcacactgggttctagtcccggtcggggcgccggattctgtcctggttgcccctcttccaggccagctctctgctgtggccagggagtgcagtggaggatggcccagctccttgggccctgcaccccatgggagaccaggagaagcacctggctcctgccttcggatcagcgcggtgcggcggcggccattggagggtgaaccaacggaaaaggaagacctttctctctgtctctctctctctcactgtccactctgcctgtcaaaaaaataaaataaaaaacccaaagctctacccggctcaagggtgaggaaaaaaaaatagcaagagaagcaacctggagagttatctctaaaatcacatggcataatgagaagagacatgatttggtgtatggggaggaagactacacagtggggacagatggagaaaactcaaacctatcatctaaaaaatcatctggggaatgaagcaaataaaggaaacaacaaatgaaaatttcagtttcattgaaaatgagcagatcaattcaactagatatgcatggcaactgtttggcagaaaaaaatcaaaataaagggtcaattataattgtatgcattttcttgatcagttacctgttgtagaattgagtctgctttaggacgaaaatcttattattttgctcattgctgcattcctagtacctggacactgacaatgaaagatgctaaataaatatttttgaatatatgaatcaatacatatttctgtaaatattgataactttatccctttcaaaaagtaaagcatggtagtgtgagtgagagagaaaatcagaagcatggaggagagtagtgaaatttgaattttataccagggaagattttgaatttgatcatctgacaaaacttctttacttttttacggtgaagtgcaagcatttttactgcattatcttggatgtcttttaaaggaacactagccctactcaagtaaaaacattgacctgattgactaattgattgactgattaattcccttgtctctccattcacag

SEQ ID NO: 3 - DNA, 23 bp, Artificial Sequence
  Synthetic
ggtcctcattctcgcctgcctgg

SEQ ID NO: 4 - DNA, 23 bp, Artificial Sequence
  Synthetic
ggtggctctcgctcttgcaaggg

SEQ ID NO: 5 - DNA, 23 bp, Artificial Sequence
  Synthetic
ggggttagggagtaggcaagagg

SEQ ID NO: 6 - DNA, 51 bp, Artificial Sequence
  Synthetic
ccatcgcctagatcatcaacccaacttgcctcttttcagtcgagtttaagg

SEQ ID NO: 7 - DNA, 23 bp, Artificial Sequence
  Synthetic
tcgactgaaaagaggcaagttgg

SEQ ID NO: 8 - DNA, 23 bp, Artificial Sequence
  Synthetic
gcaagttgggttgatgatctagg

SEQ ID NO: 9 - DNA, 23 bp, Artificial Sequence
  Synthetic
cgactgaaaagaggcaagttggg

SEQ ID NO: 10 - DNA, 34 bp, Artificial Sequence
  Synthetic
gtgccagggcgtgcccttgggctccccgggcgcg

SEQ ID NO: 11 - DNA, 39 bp, Artificial Sequence
  Synthetic
ccccaactggggtaacctttgagttctctcagttggggg

SEQ ID NO: 12 - DNA, 35 bp, Artificial Sequence
  Synthetic
gtgccagggcgtgcccttgagttctcagttggggg

SEQ ID NO: 13 - DNA, 36 bp, Artificial Sequence
  Synthetic
ccccaactggggtaacctttgggctccccgggcgcg

SEQ ID NO: 14 - DNA, 83 bp, Artificial Sequence
  Synthetic
ctatggccgtgatgacctgtgtcttcgtggtttgtctggtcaaccaccgcggtctcagtggtgtacggtacaaacccagtcga

SEQ ID NO: 15 - DNA, 78 bp, Artificial Sequence
  Synthetic
ctggccgtggccgtgctcgtcctcgtcggccggcttgtcgacgacggcggtctccgtcgtcaggatcatccgggccac

SEQ ID NO: 16 - DNA, 82 bp, Artificial Sequence
  Synthetic
ctggccgtggccgtgctcgtcctcgtcggccggcttgtcgacgacggcggtctcagtggtgtacggtacaaacccagtcgac

SEQ ID NO: 17 - DNA, 80 bp, Artificial Sequence
  Synthetic
ctatggccgtgatgacctgtgtcttcgtggtttgtctggtcaaccaccgcggtctccgtcgtcaggatcatccgggccac